European Patent Specification EP 3 922 728 B1, published November 29, 2023. Title: Production Method of (1R,3R)-3-(Trifluoromethyl)cyclohexane-1-ol and Intermediates Thereof. Applicant: API CORPORATION. The sequence listing filed with the application follows.

SEQUENCE LISTING (10 sequences)

SEQ ID NO: 1 - protein, 338 aa, Bacillus subtilis
MARKLFTPITIKDMTLKNRIVMSPMCMYSSHEKDGKLTPFHMAHYISRAIGQVGLIIVEASAVNPQGRITDQDLGIWSDEHIEGFAKLTEQVKEQGSKIGIQLAHAGRKAELEGDIFAPSAIAFDEQSATPVEMSAEKVKETVQEFKQAAARAKEAGFDVIEIHAAHGYLIHEFLSPLSNHRTDEYGGSPENRYRFLREIIDEVKQVWDGPLFVRVSASDYTDKGLDIADHIGFAKWMKEQGVDLIDCSSGALVHADINVFPGYQVSFAEKIREQADMATGAVGMITDGSMAEEILQNGRADLIFIGRELLRDPFFARTAAKQLNTEIPAPVQYERGW

SEQ ID NO: 2 - protein, 252 aa, Lactobacillus kefir
MTDRLKGKVAIVTGGTLGIGLAIADKFVEEGAKVVITGRHADVGEKAAKSIGGTDVIRFVQHDASDEAGWTKLFDTTEEAFGPVTTVVNNAGIAVSKSVEDTTTEEWRKLLSVNLDGVFFGTRLGIQRMKNKGLGASIINMSSIEGFVGDPTLGAYNASKGAVRIMSKSAALDCALKDYDVRVNTVHPGYIKTPLVDDLEGAEEMMSQRTKTPMGHIGEPNDIAWICVYLASDESKFATGAEFVVDGGYTAQ

SEQ ID NO: 3 - protein, 234 aa, Pichia finlandica
LSVAKKFLQLGAKVTISDVSGEKKYHETVVALKAQNLNTDNLHYVQADSSKEEDNKKLISETLATFGGLDIVCANAGIGKFAPTHETPFDVWKKVIAVNLNGVFLLDKLAINYWLEKSKPGVIVNMGSVHSFVAAPGLAHYGAAKGGVKLLTQTLALEYASHGIRVNSVNPGYISTPLIDEVPKERLDKLVSLHPIGRLGRPEEVADAVAFLCSQEATFINGVSLPVDGGYTAQ

SEQ ID NO: 4 - protein, 210 aa, Devosia riboflavina
LEGAQAVADAVKAAGGEAAAVAVDVAKADQVEKAVQFAVDTFGALHLAVNNAGIGGASAPLGDYSFDDWHRVIDVNLNSVFYSMKYEIVAMLRAGGGAIVNMASILGSVTFPNAPAYVTAKHGVVGMTKSAAVDYAKKGIRVTAVGPGFIDTPLLSALPKETLDYLKSVHPIGRLGTSDEVAALTAFLLSDAASNITGSYHLVDGGYVAQ

SEQ ID NO: 5 - DNA, 1017 bp, Bacillus subtilis
atggccagaaaattatttacacctattacaattaaagatatgacgttaaaaaaccgcattgtcatgtcgccaatgtgcatgtattcttctcatgaaaaggacggaaaattaacaccgttccacatggcacattacatatcgcgcgcaatcggccaggtcggactgattattgtagaggcgtcagcggttaaccctcaaggacgaatcactgaccaagacttaggcatttggagcgacgagcatattgaaggctttgcaaaactgactgagcaggtcaaagaacaaggttcaaaaatcggcattcagcttgcccatgccggacgtaaagctgagcttgaaggagatatcttcgctccatcggcgattgcgtttgacgaacaatcagcaacacctgtagaaatgtcagcagaaaaagtaaaagaaacggtccaggagttcaagcaagcggctgcccgcgcaaaagaagccggctttgatgtgattgaaattcatgcggcgcacggatatttaattcatgaatttttgtctccgctttccaaccatcgaacagatgaatatggcggctcacctgaaaaccgctatcgtttcttgagagagatcattgatgaagtcaaacaagtatgggacggtcctttatttgtccgtgtatctgcttctgactacactgataaaggcttagacattgccgatcacatcggttttgcaaaatggatgaaggagcagggtgttgacttaattgactgcagctcaggcgcccttgttcacgcagacattaacgtattccctggctatcaggtcagcttcgctgagaaaatccgtgaacaggcggacatggctactggtgccgtcggcatgattacagacggttcaatggctgaagaaattctgcaaaacggacgtgccgacctcatctttatcggcagagagcttttgcgggatccattttttgcaagaactgctgcgaaacagctcaatacagagattccggcccctgttcaatacgaaagaggctggtaa

SEQ ID NO: 6 - DNA, 759 bp, Lactobacillus kefir
atgactgatcgtttaaaaggcaaagtagcaattgtaactggcggtaccttgggaattggcttggcaatcgctgataagtttgttgaagaaggcgcaaaggttgttattaccggccgtcacgctgatgtaggtgaaaaagctgccaaatcaatcggcggcacagacgttatccgttttgtccaacacgatgcttctgatgaagccggctggactaagttgtttgatacgactgaagaagcatttggcccagttaccacggttgtcaacaatgccggaattgcggtcagcaagagtgttgaagataccacaactgaagaatggcgcaagctgctctcagttaacttggatggtgtcttcttcggtacccgtcttggaatccaacgtatgaagaataaaggactcggagcatcaatcatcaatatgtcatctatcgaaggttttgttggtgatccaactctgggtgcatacaacgcttcaaaaggtgctgtcagaattatgtctaaatcagctgccttggattgcgctttgaaggactacgatgttcgggttaacactgttcatccaggttatatcaagacaccattggttgacgatcttgaaggggcagaagaaatgatgtcacagcggaccaagacaccaatgggtcatatcggtgaacctaacgatatcgcttggatctgtgtttacctggcatctgacgaatctaaatttgccactggtgcagaattcgttgtcgatggtggatacactgctcaataa

SEQ ID NO: 7 - DNA, 765 bp, Pichia finlandica
atgtcttataacttccataacaaggttgcagttgttactggagctctatcaggaatcggcttaagcgtcgcaaaaaagttccttcagctcggcgccaaagtaacgatctctgatgtcagtggagagaaaaaatatcacgagactgttgttgctctgaaagcccaaaatctcaacactgacaacctccattatgtacaggcagattccagcaaagaagaagataacaagaaattgatttcggaaactctggcaacctttgggggcctggatattgtttgtgctaatgcaggaattggaaagttcgctcccacccatgaaacacccttcgacgtatggaagaaggtgattgctgtgaatttgaatggagtattcttactggataagctagccatcaattactggctagagaaaagcaaacccggcgtaattgtcaacatgggatcagtccactcttttgtagcagctcctggccttgcgcattatggagctgcaaaaggcggtgtcaaactgttaacacaaacattggctctagagtacgcatctcatggtattagagtaaattctgtcaatccggggtacatttcgactcctttgatagatgaggttccgaaagagcggttggataaacttgtaagcttgcaccctattgggagactaggtcgtccagaggaagttgctgatgcagtcgcatttctgtgttcccaggaggccactttcatcaacggcgtttctttgccggttgacggggggtacacagcccagtaa

SEQ ID NO: 8 - DNA, 753 bp, Devosia riboflavina
atgtcccaggatttttcaggcaaggtcgcattcgtaacgggtggtgcctcgggcatcggtgaggcggtcgtcaagcagcttgccgcgcgcggcgccaaggttgtggttgccgatctcaagctcgaaggcgcgcaggcggttgccgatgcggtcaaggccgccggcggcgaagcggccgcggtagctgtcgatgtcgccaaggccgatcaggtggagaaggctgtccagttcgccgtcgacacctttggcgccctgcatctggcggtcaataatgccggcattggcggcgcttccgctcccctcggcgattattccttcgacgactggcatagggttatcgacgtcaatctcaattccgtcttctattcgatgaagtacgagatcgtcgccatgctcagggcaggcggtggcgccatcgtcaacatggcctccatcctcggctcggtgacctttcccaatgcaccggcctatgtcaccgccaagcacggcgtggtcggcatgaccaagtcggccgcggtggactatgccaaaaagggcattcgcgtcacggccgtcgggcccggtttcatcgacacgccgctcctatccgccttgcccaaggaaaccctggactacctcaaatccgtccatccgatcggacggctgggtacctcggatgaagtcgcagcgctgaccgcgttcctgctctccgatgcagcgtcgaacatcaccggctcctatcacctggtcgatggcggctacgtcgcccaatag

SEQ ID NO: 9 - protein, 261 aa, Bacillus subtilis
MYPDLKGKVVAITGAASGLGKAMAIRFGKEQAKVVINYYSNKQDPNEVKEEVIKAGGEAVVVQGDVTKEEDVKNIVQTAIKEFGTLDIMINNAGLANPVPSHEMPLKDWDKVIGTNLTGAFLGSREAIKYFVENDIKGNVINMSSVHEVIPWPLFVHYAASKGGIKLMTETLALEYAPKGIRVNNIGPGAINTPINAEKFADPKQKADVESMIPMGYIGEPEEIAAVAAWLASKEASYVTGITLFADGGMTLYPSFQAGRG

SEQ ID NO: 10 - DNA, 786 bp, Bacillus subtilis
atgtatccggatttaaaaggaaaagtcgtcgctattacaggagctgcttcagggctcggaaaggcgatggccattcgcttcggcaaggagcaggcaaaagtggttatcaactattatagtaataaacaagatccgaacgaggtaaaagaagaggtcatcaaggcgggcggtgaagctgttgtcgtccaaggagatgtcacgaaagaggaagatgtaaaaaatatcgtgcaaacggcaattaaggagttcggcacactcgatattatgattaataatgccggtcttgcaaatcctgtgccatctcacgaaatgccgctcaaggattgggataaagtcatcggcacgaacttaacgggtgcctttttaggaagccgtgaagcgattaaatatttcgtagaaaacgatatcaagggaaatgtcattaacatgtccagtgtgcacgaagtgattccttggccgttatttgtccactatgcggcaagtaaaggcgggataaagctgatgacagaaacattagcgttggaatacgcgccgaagggcattcgcgtcaataatattgggccaggtgcgatcaacacgccaatcaatgctgaaaaattcgctgaccctaaacagaaagctgatgtagaaagcatgattccaatgggatatatcggcgaaccggaggagatcgccgcagtagcagcctggcttgcttcgaaggaagccagctacgtcacaggcatcacgttattcgcggacggcggtatgacactgtatccttcattccaggcaggccgcggttaa